European Patent Specification EP 3 280 732 B1, published October 18, 2023. Title: ANTIBODIES BINDING TO CANINE VASCULAR ENDOTHELIAL GROWTH FACTOR AND USES THEREOF IN TREATING CANINE DISEASES. Applicant: YUNG SHIN PHARMACEUTICAL INDUSTRIAL CO. LTD. Application Not yet assigned. The sequence listing filed with the application follows.

SEQUENCE LISTING (10 sequences)

SEQ ID NO: 1 - DNA, 1389 bp, Artificial Sequence
  Synthetic Polynucleotide
atggaatggacctgggtctttctcttcctcctgtcagtaactgcaggtgtccactcccaggttcagctgcagcagtctggagctgagctgatgaagcctggggcctcagtgaaaatatcctgcaaggctactggctacacattcagtagctactggatagagtgggtaaagcagaggcctggacatggccttgagtggattggagagatttttcctggaggtggtgatcctaaatacaatgagaatttcaagggcaaggccacattcactacagatgcatcctccaacacagcctacatgcaactcagcagcctgacatctgaggactctgccgtctattactgtgcaagaggaaccttcgggttctatgctatggactactggggtcaaggaacctcagtcaccgtctcctcagccaaaacgacacccccatctgtctatccactggcccctggatctgctgcccaaactaactccatggtgaccctgggatgcctggtcaagggctatttccctgagccagtgacagtgacctggaactctggatccctgtccagcggtgtgcacaccttcccagctgtcctgcagtctgacctctacactctgagcagctcagtgactgtcccctccagcacctggcccagcgagaccgtcacctgcaacgttgcccacccggccagcagcaccaaggtggacaagaaaattgtgcccagggattgtggttgtaagccttgcatatgtacagtcccagaagtatcatctgtcttcatcttccccccaaagcccaaggatgtgctcaccattactctgactcctaaggtcacgtgtgttgtggtagacatcagcaaggatgatcccgaggtccagttcagctggtttgtagatgatgtggaggtgcacacagctcagacgcaaccccgggaggagcagttcaacagcactttccgctcagtcagtgaacttcccatcatgcaccaggactggctcaatggcaaggagttcaaatgcagggtcaacagtgcagctttccctgcccccatcgagaaaaccatctccaaaaccaaaggcagaccgaaggctccacaggtgtacaccattccacctcccaaggagcagatggccaaggataaagtcagtctgacctgcatgataacagacttcttccctgaagacattactgtggagtggcagtggaatgggcagccagcggagaactacaagaacactcagcccatcatggacacagatggctcttacttcgtctacagcaagctcaatgtgcagaagagcaactgggaggcaggaaatactttcacctgctctgtgttacatgagggcctgcacaaccaccatactgagaagagcctctcccactctcctggtaaatga

SEQ ID NO: 2 - protein, 462 aa, Artificial Sequence
  Synthetic Polypeptide
MEWTWVFLFLLSVTAGVHSQVQLQQSGAELMKPGASVKISCKATGYTFSSYWIEWVKQRPGHGLEWIGEIFPGGGDPKYNENFKGKATFTTDASSNTAYMQLSSLTSEDSAVYYCARGTFGFYAMDYWGQGTSVTVSSAKTTPPSVYPLAPGSAAQTNSMVTLGCLVKGYFPEPVTVTWNSGSLSSGVHTFPAVLQSDLYTLSSSVTVPSSTWPSETVTCNVAHPASSTKVDKKIVPRDCGCKPCICTVPEVSSVFIFPPKPKDVLTITLTPKVTCVVVDISKDDPEVQFSWFVDDVEVHTAQTQPREEQFNSTFRSVSELPIMHQDWLNGKEFKCRVNSAAFPAPIEKTISKTKGRPKAPQVYTIPPPKEQMAKDKVSLTCMITDFFPEDITVEWQWNGQPAENYKNTQPIMDTDGSYFVYSKLNVQKSNWEAGNTFTCSVLHEGLHNHHTEKSLSHSPGK

SEQ ID NO: 3 - DNA, 717 bp, Artificial Sequence
  Synthetic Polynucleotide
atgaagttgcctgttaggctgttggtgctgatgttctggattcctgcttccagcagtgatgctgtgatgacccaaactccactctccctgcctgtcagtcttggagatcaagtctccatctcttgcaggtctagtcagagccttgaaaacagtaatggaaacacctatttgaactggtacctccagaaaccaggccagtctccacagctcctgatctacagggtttccaaccgattttctggggtcctagacaggttcagtggtagtggatcagggacagatttcacactgaaaatcagcagagtggaggctgaggatttgggagtttatttctgcctccaagttacacatgtcccctacacgttcggaggggggaccaagctggaaataaaacgggctgatgctgcaccaactgtatccatcttcccaccatccagtgagcagttaacatctggaggtgcctcagtcgtgtgcttcttgaacaacttctaccccaaagacatcaatgtcaagtggaagattgatggcagtgaacgacaaaatggcgtcctgaacagttggactgatcaggacagcaaagacagcacctacagcatgagcagcaccctcacgttgaccaaggacgagtatgaacgacataacagctatacctgtgaggccactcacaagacatcaacttcacccattgtcaagagcttcaacaggaatgagtgttag

SEQ ID NO: 4 - protein, 238 aa, Artificial Sequence
  Synthetic Polypeptide
MKLPVRLLVLMFWIPASSSDAVMTQTPLSLPVSLGDQVSISCRSSQSLENSNGNTYLNWYLQKPGQSPQLLIYRVSNRFSGVLDRFSGSGSGTDFTLKISRVEAEDLGVYFCLQVTHVPYTFGGGTKLEIKRADAAPTVSIFPPSSEQLTSGGASVVCFLNNFYPKDINVKWKIDGSERQNGVLNSWTDQDSKDSTYSMSSTLTLTKDEYERHNSYTCEATHKTSTSPIVKSFNRNEC

SEQ ID NO: 5 - protein, 10 aa, Artificial Sequence
  Synthetic Polypeptide
GYTFSSYWIE

SEQ ID NO: 6 - protein, 17 aa, Artificial Sequence
  Synthetic Polypeptide
EIFPGGGDPKYNENFKG

SEQ ID NO: 7 - protein, 10 aa, Artificial Sequence
  Synthetic Polypeptide
GTFGFYAMDY

SEQ ID NO: 8 - protein, 16 aa, Artificial Sequence
  Synthetic Polypeptide
RSSQSLENSNGNTYLN

SEQ ID NO: 9 - protein, 7 aa, Artificial Sequence
  Synthetic Polypeptide
RVSNRFS

SEQ ID NO: 10 - protein, 8 aa, Artificial Sequence
  Synthetic Polypeptide
LQVTHVPY